European Patent Specification EP 2 872 636 B1, published June 11, 2025. Title: METHOD FOR INDUCING CELLS TO LESS MATURE STATE. Applicant: Minerva Biotechnologies Corporation. The sequence listing filed with the application follows.

SEQUENCE LISTING (40 sequences)

SEQ ID NO: 1 - protein, 1255 aa, Artificial Sequence
  full-length MUC1 Receptor
MTPGTQSPFFLLLLLTVLTVVTGSGHASSTPGGEKETSATQRSSVPSSTEKNAVSMTSSVLSSHSPGSGSSTTQGQDVTLAPATEPASGSAATWGQDVTSVPVTRPALGSTTPPAHDVTSAPDNKPAPGSTAPPAHGVTSAPDTRPAPGSTAPPAHGVTSAPDTRPAPGSTAPPAHGVTSAPDTRPAPGSTAPPAHGVTSAPDTRPAPGSTAPPAHGVTSAPDTRPAPGSTAPPAHGVTSAPDTRPAPGSTAPPAHGVTSAPDTRPAPGSTAPPAHGVTSAPDTRPAPGSTAPPAHGVTSAPDTRPAPGSTAPPAHGVTSAPDTRPAPGSTAPPAHGVTSAPDTRPAPGSTAPPAHGVTSAPDTRPAPGSTAPPAHGVTSAPDTRPAPGSTAPPAHGVTSAPDTRPAPGSTAPPAHGVTSAPDTRPAPGSTAPPAHGVTSAPDTRPAPGSTAPPAHGVTSAPDTRPAPGSTAPPAHGVTSAPDTRPAPGSTAPPAHGVTSAPDTRPAPGSTAPPAHGVTSAPDTRPAPGSTAPPAHGVTSAPDTRPAPGSTAPPAHGVTSAPDTRPAPGSTAPPAHGVTSAPDTRPAPGSTAPPAHGVTSAPDTRPAPGSTAPPAHGVTSAPDTRPAPGSTAPPAHGVTSAPDTRPAPGSTAPPAHGVTSAPDTRPAPGSTAPPAHGVTSAPDTRPAPGSTAPPAHGVTSAPDTRPAPGSTAPPAHGVTSAPDTRPAPGSTAPPAHGVTSAPDTRPAPGSTAPPAHGVTSAPDTRPAPGSTAPPAHGVTSAPDTRPAPGSTAPPAHGVTSAPDTRPAPGSTAPPAHGVTSAPDTRPAPGSTAPPAHGVTSAPDTRPAPGSTAPPAHGVTSAPDTRPAPGSTAPPAHGVTSAPDTRPAPGSTAPPAHGVTSAPDTRPAPGSTAPPAHGVTSAPDTRPAPGSTAPPAHGVTSAPDNRPALGSTAPPVHNVTSASGSASGSASTLVHNGTSARATTTPASKSTPFSIPSHHSDTPTTLASHSTKTDASSTHHSSVPPLTSSNHSTSPQLSTGVSFFFLSFHISNLQFNSSLEDPSTDYYQELQRDISEMFLQIYKQGGFLGLSNIKFRPGSVVVQLTLAFREGTINVHDVETQFNQYKTEAASRYNLTISDVSVSDVPFPFSAQSGAGVPGWGIALLVLVCVLVALAIVYLIALAVCQCRRKNYGQLDIFPARDTYHPMSEYPTYHTHGRYVPPSSTDRSPYEKVSAGNGGSSLSYTNPAVAAASANL

SEQ ID NO: 2 - protein, 19 aa, Artificial Sequence
  N-terminal MUC-1 signaling sequence
MTPGTQSPFFLLLLLTVLT

SEQ ID NO: 3 - protein, 23 aa, Artificial Sequence
  N-terminal MUC-1 signaling sequence
MTPGTQSPFFLLLLLTVLTVVTA

SEQ ID NO: 4 - protein, 23 aa, Artificial Sequence
  N-terminal MUC-1 signaling sequence
MTPGTQSPFFLLLLLTVLTVVTG

SEQ ID NO: 5 - protein, 146 aa, Artificial Sequence
  truncated MUC1 receptor isoform
GTINVHDVETQFNQYKTEAASRYNLTISDVSVSDVPFPFSAQSGAGVPGWGIALLVLVCVLVALAIVYLIALAVCQCRRKNYGQLDIFPARDTYHPMSEYPTYHTHGRYVPPSSTDRSPYEKVSAGNGGSSLSYTNPAVAAASANL

SEQ ID NO: 6 - protein, 45 aa, Artificial Sequence
  Native Primary Sequence of the MUC1 Growth Factor Receptor
GTINVHDVETQFNQYKTEAASRYNLTISDVSVSDVPFPFSAQSGA

SEQ ID NO: 7 - protein, 44 aa, Artificial Sequence
  Native Primary Sequence of the MUC1 Growth Factor Receptor
TINVHDVETQFNQYKTEAASRYNLTISDVSVSDVPFPFSAQSGA

SEQ ID NO: 8 - protein, 45 aa, Artificial Sequence
  "SPY" functional variant of the native Primary Sequence of the MUC1 Growth Factor Receptor
GTINVHDVETQFNQYKTEAASPYNLTISDVSVSDVPFPFSAQSGA

SEQ ID NO: 9 - protein, 44 aa, Artificial Sequence
  "SPY" functional variant of the native Primary Sequence of the MUC1 Growth Factor Receptor
TINVHDVETQFNQYKTEAASPYNLTISDVSVSDVPFPFSAQSGA

SEQ ID NO: 10 - DNA, 216 bp, Artificial Sequence
  MUC1 cytoplasmic domain nucleotide sequence
tgtcagtgccgccgaaagaactacgggcagctggacatctttccagcccgggatacctaccatcctatgagcgagtaccccacctaccacacccatgggcgctatgtgccccctagcagtaccgatcgtagcccctatgagaaggtttctgcaggtaacggtggcagcagcctctcttacacaaacccagcagtggcagccgcttctgccaacttg

SEQ ID NO: 11 - protein, 72 aa, Artificial Sequence
  MUC1 cytoplasmic domain amino acid sequence
CQCRRKNYGQLDIFPARDTYHPMSEYPTYHTHGRYVPPSSTDRSPYEKVSAGNGGSSLSYTNPAVAAASANL

SEQ ID NO: 12 - DNA, 854 bp, Artificial Sequence
  NME7 nucleotide sequence
gagatcctgagacaatgaatcatagtgaaagattcgttttcattgcagagtggtatgatccaaatgcttcacttcttcgacgttatgagcttttattttacccaggggatggatctgttgaaatgcatgatgtaaagaatcatcgcacctttttaaagcggaccaaatatgataacctgcacttggaagatttatttataggcaacaaagtgaatgtcttttctcgacaactggtattaattgactatggggatcaatatacagctcgccagctgggcagtaggaaagaaaaaacgctagccctaattaaaccagatgcaatatcaaaggctggagaaataattgaaataataaacaaagctggatttactataaccaaactcaaaatgatgatgctttcaaggaaagaagcattggattttcatgtagatcaccagtcaagaccctttttcaatgagctgatccagtttattacaactggtcctattattgccatggagattttaagagatgatgctatatgtgaatggaaaagactgctgggacctgcaaactctggagtggcacgcacagatgcttctgaaagcattagagccctctttggaacagatggcataagaaatgcagcgcatggccctgattcttttgcttctgcggccagagaaatggagttgttttttccttcaagtggaggttgtgggccggcaaacactgctaaatttactaattgtacctgttgcattgttaaaccccatgctgtcagtgaaggtatgttgaatacactatattcagtacattttgttaataggagagcaatgtttattttcttgatgtactttatgtatagaaaataa

SEQ ID NO: 13 - protein, 283 aa, Artificial Sequence
  NME7 amino acid sequence
DPETMNHSERFVFIAEWYDPNASLLRRYELLFYPGDGSVEMHDVKNHRTFLKRTKYDNLHLEDLFIGNKVNVFSRQLVLIDYGDQYTARQLGSRKEKTLALIKPDAISKAGEIIEIINKAGFTITKLKMMMLSRKEALDFHVDHQSRPFFNELIQFITTGPIIAMEILRDDAICEWKRLLGPANSGVARTDASESIRALFGTDGIRNAAHGPDSFASAAREMELFFPSSGGCGPANTAKFTNCTCCIVKPHAVSEGMLNTLYSVHFVNRRAMFIFLMYFMYRK

SEQ ID NO: 14 - DNA, 534 bp, Artificial Sequence
  NM23-H1 nucleotide sequence
atggtgctactgtctactttagggatcgtctttcaaggcgaggggcctcctatctcaagctgtgatacaggaaccatggccaactgtgagcgtaccttcattgcgatcaaaccagatggggtccagcggggtcttgtgggagagattatcaagcgttttgagcagaaaggattccgccttgttggtctgaaattcatgcaagcttccgaagatcttctcaaggaacactacgttgacctgaaggaccgtccattctttgccggcctggtgaaatacatgcactcagggccggtagttgccatggtctgggaggggctgaatgtggtgaagacgggccgagtcatgctcggggagaccaaccctgcagactccaagcctgggaccatccgtggagacttctgcatacaagttggcaggaacattatacatggcagtgattctgtggagagtgcagagaaggagatcggcttgtggtttcaccctgaggaactggtagattacacgagctgtgctcagaactggatctatgaatga

SEQ ID NO: 15 - protein, 177 aa, Artificial Sequence
  NM23-H1 describes amino acid sequence
MVLLSTLGIVFQGEGPPISSCDTGTMANCERTFIAIKPDGVQRGLVGEIIKRFEQKGFRLVGLKFMQASEDLLKEHYVDLKDRPFFAGLVKYMHSGPVVAMVWEGLNVVKTGRVMLGETNPADSKPGTIRGDFCIQVGRNIIHGSDSVESAEKEIGLWFHPEELVDYTSCAQNWIYE

SEQ ID NO: 16 - DNA, 534 bp, Artificial Sequence
  NM23-H1 S120G mutant nucleotide sequence
atggtgctactgtctactttagggatcgtctttcaaggcgaggggcctcctatctcaagctgtgatacaggaaccatggccaactgtgagcgtaccttcattgcgatcaaaccagatggggtccagcggggtcttgtgggagagattatcaagcgttttgagcagaaaggattccgccttgttggtctgaaattcatgcaagcttccgaagatcttctcaaggaacactacgttgacctgaaggaccgtccattctttgccggcctggtgaaatacatgcactcagggccggtagttgccatggtctgggaggggctgaatgtggtgaagacgggccgagtcatgctcggggagaccaaccctgcagactccaagcctgggaccatccgtggagacttctgcatacaagttggcaggaacattatacatggcggtgattctgtggagagtgcagagaaggagatcggcttgtggtttcaccctgaggaactggtagattacacgagctgtgctcagaactggatctatgaatga

SEQ ID NO: 17 - protein, 177 aa, Artificial Sequence
  NM23-H1 S120G mutant amino acid sequence
MVLLSTLGIVFQGEGPPISSCDTGTMANCERTFIAIKPDGVQRGLVGEIIKRFEQKGFRLVGLKFMQASEDLLKEHYVDLKDRPFFAGLVKYMHSGPVVAMVWEGLNVVKTGRVMLGETNPADSKPGTIRGDFCIQVGRNIIHGGDSVESAEKEIGLWFHPEELVDYTSCAQNWIYE

SEQ ID NO: 18 - DNA, 954 bp, Artificial Sequence
  human SOX2 nucleotide sequence
atgtacaacatgatggagacggagctgaagccgccgggcccgcagcaaacttcggggggcggcggcggcaactccaccgcggcggcggccggcggcaaccagaaaaacagcccggaccgcgtcaagcggcccatgaatgccttcatggtgtggtcccgcgggcagcggcgcaagatggcccaggagaaccccaagatgcacaactcggagatcagcaagcgcctgggcgccgagtggaaacttttgtcggagacggagaagcggccgttcatcgacgaggctaagcggctgcgagcgctgcacatgaaggagcacccggattataaataccggccccggcggaaaaccaagacgctcatgaagaaggataagtacacgctgcccggcgggctgctggcccccggcggcaatagcatggcgagcggggtcggggtgggcgccggcctgggcgcgggcgtgaaccagcgcatggacagttacgcgcacatgaacggctggagcaacggcagctacagcatgatgcaggaccagctgggctacccgcagcacccgggcctcaatgcgcacggcgcagcgcagatgcagcccatgcaccgctacgacgtgagcgccctgcagtacaactccatgaccagctcgcagacctacatgaacggctcgcccacctacagcatgtcctactcgcagcagggcacccctggcatggctcttggctccatgggttcggtggtcaagtccgaggccagctccagcccccctgtggttacctcttcctcccactccagggcgccctgccaggccggggacctccgggacatgatcagcatgtatctccccggcgccgaggtgccggaacccgccgcccccagcagacttcacatgtcccagcactaccagagcggcccggtgcccggcacggccattaacggcacactgcccctctcacacatgtga

SEQ ID NO: 19 - protein, 317 aa, Artificial Sequence
  human SOX2 amino acid sequence
MYNMMETELKPPGPQQTSGGGGGNSTAAAAGGNQKNSPDRVKRPMNAFMVWSRGQRRKMAQENPKMHNSEISKRLGAEWKLLSETEKRPFIDEAKRLRALHMKEHPDYKYRPRRKTKTLMKKDKYTLPGGLLAPGGNSMASGVGVGAGLGAGVNQRMDSYAHMNGWSNGSYSMMQDQLGYPQHPGLNAHGAAQMQPMHRYDVSALQYNSMTSSQTYMNGSPTYSMSYSQQGTPGMALGSMGSVVKSEASSSPPVVTSSSHSRAPCQAGDLRDMISMYLPGAEVPEPAAPSRLHMSQHYQSGPVPGTAINGTLPLSHM

SEQ ID NO: 20 - DNA, 1083 bp, Homo sapiens
atggcgggacacctggcttcagattttgccttctcgccccctccaggtggtggaggtgatgggccaggggggccggagccgggctgggttgatcctcggacctggctaagcttccaaggccctcctggagggccaggaatcgggccgggggttgggccaggctctgaggtgtgggggattcccccatgccccccgccgtatgagttctgtggggggatggcgtactgtgggccccaggttggagtggggctagtgccccaaggcggcttggagacctctcagcctgagggcgaagcaggagtcggggtggagagcaactccgatggggcctccccggagccctgcaccgtcacccctggtgccgtgaagctggagaaggagaagctggagcaaaacccggaggagtcccaggacatcaaagctctgcagaaagaactcgagcaatttgccaagctcctgaagcagaagaggatcaccctgggatatacacaggccgatgtggggctcaccctgggggttctatttgggaaggtattcagccaaacgaccatctgccgctttgaggctctgcagcttagcttcaagaacatgtgtaagctgcggcccttgctgcagaagtgggtggaggaagctgacaacaatgaaaatcttcaggagatatgcaaagcagaaaccctcgtgcaggcccgaaagagaaagcgaaccagtatcgagaaccgagtgagaggcaacctggagaatttgttcctgcagtgcccgaaacccacactgcagcagatcagccacatcgcccagcagcttgggctcgagaaggatgtggtccgagtgtggttctgtaaccggcgccagaagggcaagcgatcaagcagcgactatgcacaacgagaggattttgaggctgctgggtctcctttctcagggggaccagtgtcctttcctctggccccagggccccattttggtaccccaggctatgggagccctcacttcactgcactgtactcctcggtccctttccctgagggggaagcctttccccctgtctctgtcaccactctgggctctcccatgcattcaaactga

SEQ ID NO: 21 - protein, 360 aa, Homo sapiens
MAGHLASDFAFSPPPGGGGDGPGGPEPGWVDPRTWLSFQGPPGGPGIGPGVGPGSEVWGIPPCPPPYEFCGGMAYCGPQVGVGLVPQGGLETSQPEGEAGVGVESNSDGASPEPCTVTPGAVKLEKEKLEQNPEESQDIKALQKELEQFAKLLKQKRITLGYTQADVGLTLGVLFGKVFSQTTICRFEALQLSFKNMCKLRPLLQKWVEEADNNENLQEICKAETLVQARKRKRTSIENRVRGNLENLFLQCPKPTLQQISHIAQQLGLEKDVVRVWFCNRRQKGKRSSSDYAQREDFEAAGSPFSGGPVSFPLAPGPHFGTPGYGSPHFTALYSSVPFPEGEAFPPVSVTTLGSPMHSN

SEQ ID NO: 22 - DNA, 459 bp, Artificial Sequence
  NM23-H2 nucleotide sequence
atggccaacctggagcgcaccttcatcgccatcaagccggacggcgtgcagcgcggcctggtgggcgagatcatcaagcgcttcgagcagaagggattccgcctcgtggccatgaagttcctccgggcctctgaagaacacctgaagcagcactacattgacctgaaagaccgaccattcttccctgggctggtgaagtacatgaactcagggccggttgtggccatggtctgggaggggctgaacgtggtgaagacaggccgagtgatgcttggggagaccaatccagcagattcaaagccaggcaccattcgtggggacttctgcattcaggttggcaggaacatcattcatggcagtgattcagtaaaaagtgctgaaaaagaaatcagcctatggtttaagcctgaagaactggttgactacaagtcttgtgctcatgactgggtctatgaataa

SEQ ID NO: 23 - protein, 152 aa, Artificial Sequence
  NM23-H2 amino acid sequence
MANLERTFIAIKPDGVQRGLVGEIIKRFEQKGFRLVAMKFLRASEEHLKQHYIDLKDRPFFPGLVKYMNSGPVVAMVWEGLNVVKTGRVMLGETNPADSKPGTIRGDFCIQVGRNIIHGSDSVKSAEKEISLWFKPEELVDYKSCAHDWVYE

SEQ ID NO: 24 - DNA, 1410 bp, Artificial Sequence
  KLF4 nucleotide sequence
atggctgtcagcgacgcgctgctcccatctttctccacgttcgcgtctggcccggcgggaagggagaagacactgcgtcaagcaggtgccccgaataaccgctggcgggaggagctctcccacatgaagcgacttcccccagtgcttcccgccggcccctatgacctggcggcggcgaccgtggccacagacctggagagcgccggagccggtgcggcttgcggcggtagcaacctggcgcccctacctcggagagagaccgaggagttcaacgatctcctggacctggactttattctctccaattcgctgacccatcctccggagtcagtggccgccaccgtgtcctcgtcagcgtcagcctcctcttcgtcgtcgccgtcgagcagcggccctgccagcgcgccctccacctgcagcttcacctatccgatccgggccgggaacgacccgggcgtggcgccgggcggcacgggcggaggcctcctctatggcagggagtccgctccccctccgacggctcccttcaacctggcggacatcaacgacgtgagcccctcgggcggcttcgtggccgagctcctgcggccagaattggacccggtgtacattccgccgcagcagccgcagccgccaggtggcgggctgatgggcaagttcgtgctgaaggcgtcgctgagcgcccctggcagcgagtacggcagcccgtcggtcatcagcgtcacgaaaggcagccctgacggcagccacccggtggtggtggcgccctacaacggcgggccgccgcgcacgtgccccaagatcaagcaggaggcggtctcttcgtgcacccacttgggcgctggaccccctctcagcaatggccaccggccggctgcacacgacttccccctggggcggcagctccccagcaggactaccccgaccctgggtcttgaggaagtgctgagcagcagggactgtcaccctgccctgccgcttcctcccggcttccatccccacccggggcccaattacccatccttcctgcccgatcagatgcagccgcaagtcccgccgctccattaccaagagctcatgccacccggttcctgcatgccagaggagcccaagccaaagaggggaagacgatcgtggccccggaaaaggaccgccacccacacttgtgattacgcgggctgcggcaaaacctacacaaagagttcccatctcaaggcacacctgcgaacccacacaggtgagaaaccttaccactgtgactgggacggctgtggatggaaattcgcccgctcagatgaactgaccaggcactaccgtaaacacacggggcaccgcccgttccagtgccaaaaatgcgaccgagcattttccaggtcggaccacctcgccttacacatgaagaggcatttt

SEQ ID NO: 25 - protein, 470 aa, Artificial Sequence [sequence omitted]

SEQ ID NO: 26 - DNA, 1362 bp, Artificial Sequence
  c-Myc nucleotide sequence
atggatttttttcgggtagtggaaaaccagcagcctcccgcgacgatgcccctcaacgttagcttcaccaacaggaactatgacctcgactacgactcggtgcagccgtatttctactgcgacgaggaggagaacttctaccagcagcagcagcagagcgagctgcagcccccggcgcccagcgaggatatctggaagaaattcgagctgctgcccaccccgcccctgtcccctagccgccgctccgggctctgctcgccctcctacgttgcggtcacacccttctcccttcggggagacaacgacggcggtggcgggagcttctccacggccgaccagctggagatggtgaccgagctgctgggaggagacatggtgaaccagagtttcatctgcgacccggacgacgagaccttcatcaaaaacatcatcatccaggactgtatgtggagcggcttctcggccgccgccaagctcgtctcagagaagctggcctcctaccaggctgcgcgcaaagacagcggcagcccgaaccccgcccgcggccacagcgtctgctccacctccagcttgtacctgcaggatctgagcgccgccgcctcagagtgcatcgacccctcggtggtcttcccctaccctctcaacgacagcagctcgcccaagtcctgcgcctcgcaagactccagcgccttctctccgtcctcggattctctgctctcctcgacggagtcctccccgcagggcagccccgagcccctggtgctccatgaggagacaccgcccaccaccagcagcgactctgaggaggaacaagaagatgaggaagaaatcgatgttgtttctgtggaaaagaggcaggctcctggcaaaaggtcagagtctggatcaccttctgctggaggccacagcaaacctcctcacagcccactggtcctcaagaggtgccacgtctccacacatcagcacaactacgcagcgcctccctccactcggaaggactatcctgctgccaagagggtcaagttggacagtgtcagagtcctgagacagatcagcaacaaccgaaaatgcaccagccccaggtcctcggacaccgaggagaatgtcaagaggcgaacacacaacgtcttggagcgccagaggaggaacgagctaaaacggagcttttttgccctgcgtgaccagatcccggagttggaaaacaatgaaaaggcccccaaggtagttatccttaaaaaagccacagcatacatcctgtccgtccaagcagaggagcaaaagctcatttctgaagaggacttgttgcggaaacgacgagaacagttgaaacacaaacttgaacagctacggaactcttgtgcg

SEQ ID NO: 27 - protein, 454 aa, Artificial Sequence
  c-Myc amino acid sequence
MDFFRVVENQQPPATMPLNVSFTNRNYDLDYDSVQPYFYCDEEENFYQQQQQSELQPPAPSEDIWKKFELLPTPPLSPSRRSGLCSPSYVAVTPFSLRGDNDGGGGSFSTADQLEMVTELLGGDMVNQSFICDPDDETFIKNIIIQDCMWSGFSAAAKLVSEKLASYQAARKDSGSPNPARGHSVCSTSSLYLQDLSAAASECIDPSVVFPYPLNDSSSPKSCASQDSSAFSPSSDSLLSSTESSPQGSPEPLVLHEETPPTTSSDSEEEQEDEEEIDVVSVEKRQAPGKRSESGSPSAGGHSKPPHSPLVLKRCHVSTHQHNYAAPPSTRKDYPAAKRVKLDSVRVLRQISNNRKCTSPRSSDTEENVKRRTHNVLERQRRNELKRSFFALRDQIPELENNEKAPKVVILKKATAYILSVQAEEQKLISEEDLLRKRREQLKHKLEQLRNSCA

SEQ ID NO: 28 - DNA, 627 bp, Artificial Sequence
  LIN28 nucleotide sequence
atgggctccgtgtccaaccagcagtttgcaggtggctgcgccaaggcggcagaagaggcgcccgaggaggcgccggaggacgcggcccgggcggcggacgagcctcagctgctgcacggtgcgggcatctgtaagtggttcaacgtgcgcatggggttcggcttcctgtccatgaccgcccgcgccggggtcgcgctcgaccccccagtggatgtctttgtgcaccagagtaagctgcacatggaagggttccggagcttgaaggagggtgaggcagtggagttcacctttaagaagtcagccaagggtctggaatccatccgtgtcaccggacctggtggagtattctgtattgggagtgagaggcggccaaaaggaaagagcatgcagaagcgcagatcaaaaggagacaggtgctacaactgtggaggtctagatcatcatgccaaggaatgcaagctgccaccccagcccaagaagtgccacttctgccagagcatcagccatatggtagcctcatgtccgctgaaggcccagcagggccctagtgcacagggaaagccaacctactttcgagaggaagaagaagaaatccacagccctaccctgctcccggaggcacagaat

SEQ ID NO: 29 - protein, 209 aa, Artificial Sequence
  LIN28 amino acid sequence
MGSVSNQQFAGGCAKAAEEAPEEAPEDAARAADEPQLLHGAGICKWFNVRMGFGFLSMTARAGVALDPPVDVFVHQSKLHMEGFRSLKEGEAVEFTFKKSAKGLESIRVTGPGGVFCIGSERRPKGKSMQKRRSKGDRCYNCGGLDHHAKECKLPPQPKKCHFCQSISHMVASCPLKAQQGPSAQGKPTYFREEEEEIHSPTLLPEAQN

SEQ ID NO: 30 - DNA, 1746 bp, Artificial Sequence
  MMP14 nucleotide sequence
atgtctcccgccccaagaccctcccgttgtctcctgctccccctgctcacgctcggcaccgcgctcgcctccctcggctcggcccaaagcagcagcttcagccccgaagcctggctacagcaatatggctacctgcctcccggggacctacgtacccacacacagcgctcaccccagtcactctcagcggccatcgctgccatgcagaagttttacggcttgcaagtaacaggcaaagctgatgcagacaccatgaaggccatgaggcgcccccgatgtggtgttccagacaagtttggggctgagatcaaggccaatgttcgaaggaagcgctacgccatccagggtctcaaatggcaacataatgaaatcactttctgcatccagaattacacccccaaggtgggcgagtatgccacatacgaggccattcgcaaggcgttccgcgtgtgggagagtgccacaccactgcgcttccgcgaggtgccctatgcctacatccgtgagggccatgagaagcaggccgacatcatgatcttctttgccgagggcttccatggcgacagcacgcccttcgatggtgagggcggcttcctggcccatgcctacttcccaggccccaacattggaggagacacccactttgactctgccgagccttggactgtcaggaatgaggatctgaatggaaatgacatcttcctggtggctgtgcacgagctgggccatgccctggggctcgagcattccagtgacccctcggccatcatggcacccttttaccagtggatggacacggagaattttgtgctgcccgatgatgaccgccggggcatccagcaactttatgggggtgagtcagggttccccaccaagatgccccctcaacccaggactacctcccggccttctgttcctgataaacccaaaaaccccacctatgggcccaacatctgtgacgggaactttgacaccgtggccatgctccgaggggagatgtttgtcttcaaggagcgctggttctggcgggtgaggaataaccaagtgatggatggatacccaatgcccattggccagttctggcggggcctgcctgcgtccatcaacactgcctacgagaggaaggatggcaaattcgtcttcttcaaaggagacaagcattgggtgtttgatgaggcgtccctggaacctggctaccccaagcacattaaggagctgggccgagggctgcctaccgacaagattgatgctgctctcttctggatgcccaatggaaagacctacttcttccgtggaaacaagtactaccgtttcaacgaagagctcagggcagtggatagcgagtaccccaagaacatcaaagtctgggaagggatccctgagtctcccagagggtcattcatgggcagcgatgaagtcttcacttacttctacaaggggaacaaatactggaaattcaacaaccagaagctgaaggtagaaccgggctaccccaagtcagccctgagggactggatgggctgcccatcgggaggccggccggatgaggggactgaggaggagacggaggtgatcatcattgaggtggacgaggagggcggcggggcggtgagcgcggctgccgtggtgctgcccgtgctgctgctgctcctggtgctggcggtgggccttgcagtcttcttcttcagacgccatgggacccccaggcgactgctctactgccagcgttccctgctggacaaggtc

SEQ ID NO: 31 - protein, 582 aa, Artificial Sequence
  MMP14 amino acid sequence
MSPAPRPSRCLLLPLLTLGTALASLGSAQSSSFSPEAWLQQYGYLPPGDLRTHTQRSPQSLSAAIAAMQKFYGLQVTGKADADTMKAMRRPRCGVPDKFGAEIKANVRRKRYAIQGLKWQHNEITFCIQNYTPKVGEYATYEAIRKAFRVWESATPLRFREVPYAYIREGHEKQADIMIFFAEGFHGDSTPFDGEGGFLAHAYFPGPNIGGDTHFDSAEPWTVRNEDLNGNDIFLVAVHELGHALGLEHSSDPSAIMAPFYQWMDTENFVLPDDDRRGIQQLYGGESGFPTKMPPQPRTTSRPSVPDKPKNPTYGPNICDGNFDTVAMLRGEMFVFKERWFWRVRNNQVMDGYPMPIGQFWRGLPASINTAYERKDGKFVFFKGDKHWVFDEASLEPGYPKHIKELGRGLPTDKIDAALFWMPNGKTYFFRGNKYYRFNEELRAVDSEYPKNIKVWEGIPESPRGSFMGSDEVFTYFYKGNKYWKFNNQKLKVEPGYPKSALRDWMGCPSGGRPDEGTEEETEVIIIEVDEEGGGAVSAAAVVLPVLLLLLVLAVGLAVFFFRRHGTPRRLLYCQRSLLDKV

SEQ ID NO: 32 - DNA, 1821 bp, Artificial Sequence
  MMP16 nucleotide
atgatcttactcacattcagcactggaagacggttggatttcgtgcatcattcgggggtgtttttcttgcaaaccttgctttggattttatgtgctacagtctgcggaacggagcagtatttcaatgtggaggtttggttacaaaagtacggctaccttccaccgactgaccccagaatgtcagtgctgcgctctgcagagaccatgcagtctgccctagctgccatgcagcagttctatggcattaacatgacaggaaaagtggacagaaacacaattgactggatgaagaagccccgatgcggtgtacctgaccagacaagaggtagctccaaatttcatattcgtcgaaagcgatatgcattgacaggacagaaatggcagcacaagcacatcacttacagtataaagaacgtaactccaaaagtaggagaccctgagactcgtaaagctattcgccgtgcctttgatgtgtggcagaatgtaactcctctgacatttgaagaagttccctacagtgaattagaaaatggcaaacgtgatgtggatataaccattatttttgcatctggtttccatggggacagctctccctttgatggagagggaggatttttggcacatgcctacttccctggaccaggaattggaggagatacccattttgactcagatgagccatggacactaggaaatcctaatcatgatggaaatgacttatttcttgtagcagtccatgaactgggacatgctctgggattggagcattccaatgaccccactgccatcatggctccattttaccagtacatggaaacagacaacttcaaactacctaatgatgatttacagggcatccagaaaatatatggtccacctgacaagattcctccacctacaagacctctaccgacagtgcccccacaccgctctattcctccggctgacccaaggaaaaatgacaggccaaaacctcctcggcctccaaccggcagaccctcctatcccggagccaaacccaacatctgtgatgggaactttaacactctagctattcttcgtcgtgagatgtttgttttcaaggaccagtggttttggcgagtgagaaacaacagggtgatggatggatacccaatgcaaattacttacttctggcggggcttgcctcctagtatcgatgcagtttatgaaaatagcgacgggaattttgtgttctttaaaggtaacaaatattgggtgttcaaggatacaactcttcaacctggttaccctcatgacttgataacccttggaagtggaattccccctcatggtattgattcagccatttggtgggaggacgtcgggaaaacctatttcttcaagggagacagatattggagatatagtgaagaaatgaaaacaatggaccctggctatcccaagccaatcacagtctggaaagggatccctgaatctcctcagggagcatttgtacacaaagaaaatggctttacgtatttctacaaaggaaaggagtattggaaattcaacaaccagatactcaaggtagaacctggacatccaagatccatcctcaaggattttatgggctgtgatggaccaacagacagagttaaagaaggacacagcccaccagatgatgtagacattgtcatcaaactggacaacacagccagcactgtgaaagccatagctattgtcattccctgcatcttggccttatgcctccttgtattggtttacactgtgttccagttcaagaggaaaggaacaccccgccacatactgtactgtaaacgctctatgcaagagtgggtg

SEQ ID NO: 33 - protein, 607 aa, Artificial Sequence [sequence omitted]

SEQ ID NO: 34 - DNA, 861 bp, Artificial Sequence
  NME7-AB nucleotide sequence
atggaaaaaacgctggccctgattaaaccggatgcaatctccaaagctggcgaaattatcgaaattatcaacaaagcgggtttcaccatcacgaaactgaaaatgatgatgctgagccgtaaagaagccctggattttcatgtcgaccaccagtctcgcccgtttttcaatgaactgattcaattcatcaccacgggtccgattatcgcaatggaaattctgcgtgatgacgctatctgcgaatggaaacgcctgctgggcccggcaaactcaggtgttgcgcgtaccgatgccagtgaatccattcgcgctctgtttggcaccgatggtatccgtaatgcagcacatggtccggactcattcgcatcggcagctcgtgaaatggaactgtttttcccgagctctggcggttgcggtccggcaaacaccgccaaatttaccaattgtacgtgctgtattgtcaaaccgcacgcagtgtcagaaggcctgctgggtaaaattctgatggcaatccgtgatgctggctttgaaatctcggccatgcagatgttcaacatggaccgcgttaacgtcgaagaattctacgaagtttacaaaggcgtggttaccgaatatcacgatatggttacggaaatgtactccggtccgtgcgtcgcgatggaaattcagcaaaacaatgccaccaaaacgtttcgtgaattctgtggtccggcagatccggaaatcgcacgtcatctgcgtccgggtaccctgcgcgcaatttttggtaaaacgaaaatccagaacgctgtgcactgtaccgatctgccggaagacggtctgctggaagttcaatactttttcaaaattctggataattga

SEQ ID NO: 35 - protein, 286 aa, Artificial Sequence
  NME7-AB amino acid sequence
MEKTLALIKPDAISKAGEIIEIINKAGFTITKLKMMMLSRKEALDFHVDHQSRPFFNELIQFITTGPIIAMEILRDDAICEWKRLLGPANSGVARTDASESIRALFGTDGIRNAAHGPDSFASAAREMELFFPSSGGCGPANTAKFTNCTCCIVKPHAVSEGLLGKILMAIRDAGFEISAMQMFNMDRVNVEEFYEVYKGVVTEYHDMVTEMYSGPCVAMEIQQNNATKTFREFCGPADPEIARHLRPGTLRAIFGKTKIQNAVHCTDLPEDGLLEVQYFFKILDN

SEQ ID NO: 36 - protein, 72 aa, Homo sapiens
GGFLGLSNIKFRPGSVVVQLTLAFREGTINVHDVETQFNQYKTEAASRYNLTISDVSVSDVPFPFSAQSGAC

SEQ ID NO: 37 - protein, 35 aa, Artificial Sequence
  "N-10"
QFNQYKTEAASRYNLTISDVSVSDVPFPFSAQSGA

SEQ ID NO: 38 - protein, 35 aa, Artificial Sequence
  amino sequence encompassing N-terminal adjacent portion
GTINVHDVETQFNQYKTEAASRYNLTISDVSVSDV

SEQ ID NO: 39 - protein, 26 aa, Artificial Sequence
  self-aggregation domain of MUC1
GGFLGLSNIKFRPGSVVVQLTLAFRE

SEQ ID NO: 40 - protein, 31 aa, Artificial Sequence
  irrelevant peptide
HHHHHHSSSSGSSSSGSSSSGGRGDSGRGDS